European Patent Specification EP 3 394 244 B1, published October 11, 2023. Title: Novel EPS Gene Cluster of Texturizing Lactic Acid Bacteria. Applicant: Chr. Hansen A/S. The sequence listing filed with the application follows.

SEQUENCE LISTING (30 sequences)

SEQ ID NO: 1 - DNA, 13097 bp, Lactococcus lactis subsp. lactis
  Full EPS operon sequence
atgaatgatttgttttaccatcgtctaaaggaactagttgaatcaagtggtaaatctgcaaatcaaatagagagggaattgggttaccctagaaattctttgaataattataagttaggaggagaaccctctgggacaagattaataggactatcggagtattttagtgtgtctccaaaatatctgatgggtataattgatgagcctaatgatagttctgcaattaatctttttaaaagtctaactcaagaagagaaaaaagaaatgtgtataatttgtcaaaaatggctttttttagaatatcaaatagaattataacaataataaatttagggagtttttcttattactatgatgaaaaaaggaatttttgtaattactatagtgatatctatagcattgataattggaggtttttatagttataattctaggataaataatctttcaaaaactaataacggaaaagaagttgtaaaaaatagcagtgaaaaaaatcagatagaacttacctataaaaagtattataaaaatttaccaaaatcagttcaaaataaaatagatgatatttcatccaaaaataaagaagttactttaacttgtatttggcaatctgattcagttatttctgaacaatttcaacaaaacttacaaaaatattatggaaataagttttggaacatcaaaaatatcacttacaatggcgaaactagtgaacaattattggctgaaaaagttgaaaatcaagtattagccactaatcctgatgttgttttatatgaagctccactttttaatgataaccaaaacattgaagcaacagcctcactgactagtaatgagcaacttataacaaatttggctagtgcaggagcggaggtaatagttcaaccctctccaccgatctatggtggtgttgtgtaccccgtacaagaagaacaatttaaacaatctttatctacaaagtatccctatatagactactgggctagttacccagacaaaaattctgatgaaatgaaggggctgttttctgataatggagtatatagaacattaaatgcttcggggaataaggtttggctagattatattactaaatattttacagcaaactaattaagttataaataacaattattaaatattggagaagaaatgcaggaaacacaggaacaaacgattgatttaagagggatttttaaaattattcgcaaaaggttaggtttaatattatttagtgctttaatagtcacaatattagggagcatctacacattttttatagcctccccagtttacacagcctcaactcaacttgtcgttaaactaccaaattcggataattcagcagcctacgctggacaagtgaccgggaatattcaaatggcgaacacaattaaccaagttattgttagtccagtcattttagataaagttcaaagtaatttaaatctatctgatgactctttccaaaaacaagttacagcagcaaatcaaacaaattcacaagtcattacgcttactgttaaatattctaatccttacgttgctcaaaagattgcagacgagactgctaaaatatttagttcagacgcagcgaaactattgaatgttactaacgttaatattctatccaaagcaaaagctcaaacaacacccattagtcctaaacctaaattgtatttagcaatatctgttatagccggattagttttaggtttagccattgctttattgaaggaattgtttgataacaaaattaataaagaagaagatattgaagctctgggactcacggttcttggtgtaacaacctatgctcaaatgagtgattttaataagaatacgaataaaaatggcacgcaatcgggaactaagtcaagtccgcctagcgaccatgaagtaaatagatcatcaaaaaggaataaaagataggagttcaggatggctaaaaataaaagaagcatagacaacaatcgttatattattaccagtgtcaatcctcaatcacctatttccgaacaatatcgtacgattcgtacgaccattgattttaaaatggcggatcaagggattaaaagttttctagtaacatcttcagaagcagctgcaggtaaatcaaccgtaagtgctaatctagctgttgcttttgcacaacaaggtaaaaaagtacttttaattgatggcgatcttcgtaaaccgactgttaacattacttttaaagtacaaaatagagtaggattaaccaatattttaatgcatcaatcttcgattgaagatgccatacaagggacaagactttctgaaaatcttacaataattacctctggtccaattccacctaatccatcggaattattagcatctagtgcaatgaagaatttgattgactctgtgtccgattcctttgatattgttttgattgatactccacctctctctgcagttactgatgctcaaattttgagtatttatgtaggaggagtggttcttgttgtacgtgcctatgaaacaaaaaaagagagtttagcaaaaacaaaaaaaatactggaacaagttaatgtaaatatattaggagttgttttgcatggggtagactcttctgagtcaccgtcgtattactactacggagtagagtaattggaataaattttaatcaaataaaagacagaaatttgtagaagaggggagcaaatgattgatattcattgccatattttaccggggatagatgatggagctaaaacttctggtgatactctgacaatgctgaaatcagcaattgatgaagggataacagctatcactgcaactcctcatcataatcctcaatttaataatgaatcaccgcttattttgaaaaaagttaaggaagttcaaaatatcattgacgaacatcaattaccaattgaagttttacccggacaagaggtgagaatatatggtgatttattaaaagaattttctgaagggaagttactgacagcagcgggcacttcaagttatatactgattgaatttccatcaaatcatgtgccagcttatgctaaagaacttttttataatattcaattggagggacttcaacctattttggttcaccctgagcgtaatagtgcaatcattgagaaccctgatatattatttgattttattgaacaaggagtactaagtcagataacagcttcaagtgtcactggtcattttggtaaaaaaatacaaaagctgtcatttaaaatgatagaaaaccatctgacgcattttgttgcatcagatgcgcataatgtgacgtcacgtgcatttaagatgaaggaagcatttgaaatgattgaagatagttatggttctggtgtatcacgaaggtttaaagataatgcagagtcagtgattttaaacgaaagtttttatcaagaaaaaccaacaaagatcaaaacaaaaaaatttttaggattattttaaagggattaaaaggagtaaataatggaagtttttgaggatgcctcatcacctgaatcggaagaacacaaattagtagtattaaaaaatttttcttatggagagctgattataaaaagagcaattgatatcctaggaggattagcgggttcagttttatttcttatcgcggctgcattgctttatgtcccttacaaaatgagctcggaaaaagatcaagggccaatgttctataaacaaaaacgggttggaaaaaacggtaaaattttttatattttgaaatttagaacaatgataattaatgctgagcagtatctagagctacatccagaagttaaagccgcctatcatgccaatggtaataaactagaaaatgatccccgtgtgacgaagattggttcatttattagacaatactcagttgatgaattaccacaatttatcaatgtccttaaaggagatatggcattagtcggtccaaggccaattcaacattttgaagcgaaagaatttggggagcgcctcccttatttactgatatgtaaacctggaattactggttattggacaacacatggtcgcagtaaagctccttttcctcaacgagcagatttagaactctattatctccaatatcacagcaccaagaatgatgtcaagcttcttatgcttacaattgcacaaattattcacggatcggacgcatattaaaaaacaatgaaaaaaaagaaattattactaataagtcaaagcggaagaggtggagtaaggaaacatctttgtgatttacttacttctcttgattataaaaaatttgagatttggattgcctataatgatgatgaggtcgatgagatttttaaatatacgttggaaagtttaaggggaaaagttaaaccaatcattataaaagaaatggttagagaacttaatcctaaacaagattggattgcatttaagaaaattcgtaggtcaataaaagagataaaaccagatattgttcattgccatagttcgaaagcgggaatattagggcgagcagctgcaaaaatagtgggtataaaacaaatatattacacacctcacgcttactcttttctcgctacagaattttcagtaaaaaagaaaagattattcattaatctagaacgtttttttagtcattatgctacaactttaacatttaccgtgtcagaaggtgaaaaagaagcagcactaaaaaacaaagttgatagcaatgagaaatttaaagtaatttataatggattgaaagatataaaaatcttatctaaaatagaagccagggaaaaacttggattaccacaagataaatttatttttggtaatattgctcgaatttgtgaacaaaaaaatccaatttattttatagaagttgctcaaaaaaatcctgattattattttgtttggattggtgatggtgaacttcgtgagaaagtcaaacaagaaattctctatagaaacctgaaaaatatttgtttcttaggaaatagaaatgatgcaggaataatggtcgcggcattcgatgtgtttatatctacttctaaatatgaaggactgccctattcacctattgaagctctccgagctggagtgcctgttttgttaagtgatgttgttggtaataatgaagttgtcttaagccatagaaatggggaagtttttgatttaaattcgtctaattggaataaaagacttgatgaatttagaaagtggcaaaagaagaaaacgagtatagagatcagacaaacgtttcttaatcacttctcattggataaatcgataaaagaactaactaagatatatttgaataatgagtaataggcaacagttacatagctattttcatccaacaagtgattctatggctttcctatgatcaacaaatttagtagttatgttttattgtagcctaatattccaaaacaatttaaaacattaaaattcaagtaactttttagttaattaaattcggataggcttaataaaattgtggattaaattaacttatatgcagattctactgagattagggtcatgatcgcttgtattaattatttcacacataaccaggagtaagatttatgcttatttattttcttttatttcctataattattttattatatatttttacaaacaacggactattaaagagtaaaaaaatatttataggactttcattctccatactagggattatttcgtctatacgttctcctcaagtaggaaccgatacatcaacttaccaaacacttttcttctatcaaatacatggaataaaaatattcaattcaaacaatccggagttaagcagcaaagctccactttatggtgtatatagtcgtattgtaagtatgatttcagtaaatttacagaccattactatagctaattcattgctgatagcattcttatttggaatttttatttatagattgaaaattaatccgctatattcaactttattatttattagtattggatttttcacaagttctcttaatacatctcgacagtttatcgctatcggtttagtatgcaatgctctgctatttctatttgataaaaaggcatttatatattttgctttaatcacattagcaatatctattcatacgctagcaatagttggattgatattttatccgatttataagattaaatggacagcagtaaaaatatcctgttttctaattgtgttgacaatgacaagctttttccttgagtctgtttcgaaaatttttattcaatttttccccaattacgctttttacttacaaaatcccgtgacattctttggtgcttctagccgtataataatgattttagatattggactaattttaattattttattattttatgcgttgactaaatactatcatattaagtgtagtcaagaagaagtttctttgcttatcattttcttaattggaccattttttgaaatacttgtatttcacaatcagagtatattacttttgactcaacgatttctaacttttttttctattttaagtattgctgtaattccaggaatgtgtgctaaagtttcaaaaaaattcaataacccagaaaatgtgagttttgctttttttagtgttatatttattttcacattatttactttttctgtagaaattcaaaaatattggggagttattccctatattacttttatgtaattagaaaggtttatttaaatatgctaatttctgtaataattccaatgtataatagaaaatttacaataaagagagctatgaacagtgtactttctcaagtaccaaataaaaaggagtttcaaattgaattaattgttgttgatgactgctccactgacaatagtgttgaggttgctagagaaataaaggatgaacgggtaaaaattgtcaaacttgataaaaactcgggtgctaatgttgcgagaaattatggaattaatttagcaaatggtgagataatcgcttttaatgattcagatgatgaatggcttcctgaaaaactttctaagcaacttgaagtacttcaagaaaaaaatatagattttttgtgctgtaatatggaaacggatgtttacagtggaaaaatgaaaatgcttacgcctagaccgtcaggttttgttccaattgaagaattgcttggaaaaaattatatagtaagtactcagaatttgattggaaaagctgatatgtttaaatctaatcaattcagtcatgaaatctctcgttttcaagactgggagcttattctacggcttttgattaaggggtataggctttattttatggaagaagtattagtgagacagtatattcaaccaaatagtttatccaaaaatttaaaaaatggtgttttgtctctccgatatatgcttgaggaattcaaagaagagtatgcacagcatcctttacaaaaggcagaggtaatattaactgttggtagccatttacacaatatgaattatcgatgtgctcaattttattttaaatctttgaagttaagatttagcatgactgtattggcaaaagcactttttatgttttttacggacttatcaagaaagaaggaaagcgaatgacagagaggattacagtgattctttccgcatataacggtgagaaatatattcaaagtcaaatagacagtatacttaatcaaacatatgataattttattttatatattagagatgatggatcaactgacggaactcgaaaaattctgaagcaatattctgaaaaagattcacgagtgaaagttcaatatggtgaaaacataggctatgtaaaaagtttttttaaaatgctttctgaagtcaattcggaatatatagcattttctgatcaagatgatatttggctgcctgaaaagttatcagtcgctcaagcagctttatcacagaaaaataagagcgttcctctcatgtgggcctcaaatatatatatatgtgatgaaaaaatgaatgtaatttcgattggtgcaaggaagagaatgagtaatttctcaaattctctttttatgtgtaatactcaaggaatgacaatgataattaataataaagctagagaaaaggttgtttctaatctaccaaaacaaaatatcatgtaccacgattggtggatttatcgcgttgttagtgctttcggagaagttatatttgattcagatccatatgtaaagtatagaagacatgataaaaatgaatctgatatttcatataattttgtgaataaagtcactaatatgatgaaccgcttaataaatagcgatatgtatatacgtacgaagaaagagacacaagaatttaaaataatttttgattcacaactttcacaatcaaatagagatgtattaagtttatttgcctcaccaaaaagaaaaattcaaaaagtcttctactcaggtagattcaaaaattccgtattagatgaactagtacttcgcttattttttcttttagacattttataattaaaaaattttttaatagttatacattataagataagttgtttgtatagtactttaatggtattaaattatagaggtaagctattagacgagaatttttttattttacaacttggaaaacagactctaacaaggggaaatgagaaataaatgaataataaattaagagaaggttttacttttacagcaattggtacatatagtaattttttaattcaaattattgtacaagcaattttaagtcgattattatcgccaagagagtatggaataattgctatcatgcaagtttttatagttttttttgcaatgctggtggaagcaggaatgggacctgctatcatacaaaataaaaagttaacaaacagagacaatatgaatttatttaacttttcagctattttttctattatatttgcgattatatttggttttttaggattattacttacaaagatatatatgaatccagcatacacttacttaacttggattcagtctatttcaatattatttattgggttaaatattgttccgactgcactccttaataaaagaaaacaattcaaagctgtaaattttagtacagtagtaggggggatactatcgggagtagtcggagttacaatggctttcctgggatttggtatttattcactaattgcaagtgccattacaacggcatttgtaagtttttgcttaaacaggtattttgctaatatttggtttactaaaaattggaataaatcttctttgatttctatttggactgtttcgcggaatcagtttggaacaaattttataaattatttttcgaataattcagacaatattttagtaggaaaatttatgggagatacagcactagctaattacaataagtcttatcaactgttaacaatccctaccactttattgttgaatatagttaatccagttttacaaccaattctctcagattatcaagatgatgttgtaactataagaaaaacatactataatattgttcacttattggctctcatcgggattcctacatcaatttttcttagtatgtctgcaaaacaaattatttttttcttttttggaagtcagtgggaagaagcagtagttcccttctcttacttagcagttattgtatggtgtcaaatgacaacatattcaaatggagcaatctggcagtccagaaataaaacaaattattttcttttttcaagtgttatcaatacttttattataattttttctatcataataggtatcataataggaaatataaatgcggttgctttatttgttgcaataggaaattttataagttttttttggaaattctactatattactaaaaatgcattagaagattctataagaaatctactaaagattttcatccatcctatttttttaggattcatcacatttattgggattagattagagattttaattgatcctagaaataatttttttagtctacttctaagaagcttagtatttttttctattctaattacctatattatgtttacatctgaaaagaaaataattgaagaaatttttgataaatagtcaatgcatctataagatactaaaggattccaaaaatatataaggagaaaaacatgaaaatagcagttgttgggacaggctatgtcggtttgtctatttcagtgcttctagcacaacatcatgaagttgttgctttggatattgttgaggcgaaagtagatttgattaactctaaaaaatcgcctattgttgataaggagattgagggatttttagcaagtaaagaattaaatttacttgcgacgacggatacggctcaagcgctaaatagagctgactttgtggtcattgcaacacctaccaattatgatgatgtcaagaattattttaatacggattctgtagaagcagtaattgaagaagtttggaaatttagcccaaatgctatgattgttataaaatcaactattccagttggttttgtggaaaaaatgcgtgctaaatatgatattgataacattatcttttctccagaatttttacgagaaggtcgagcattgtatgacaatcttcatccatctcgcattgttgtgggggaacaatctgagcgtgcctctcaatttgctgagcttttaatagagggagctattgataaagatatcccagttctttttacaaaccctactgaagcagaagcgattaagctattttcaaatacatatttagctttacgcgtggcttattttaatgaattagatacttatgctgaagttcgtggtttagatacaaaacaaatcattgatggcgttggattagatccacgaattggaacacactacaataatccttcatttggttatggagggtattgcctaccgaaagataccaaacagcttttagctaactacgaccaagttcctgaaaaattaattgaggctgttgttgaatcaaatagtacaagaaaagatcatattgcagatatgatcattaaacgttctcctaaagtggtgggtatctaccgcttgactatgaagtcaaattctgataattttagatcaagttcaattcaaggaattatgaaacgaattaagggcaagggaattgaagtagttgtctatgagccaacactaaatgatactcatttctacaattctcgggtagttcataatttggatgagtttaaaacgatttctgatgtgattgtttcaaatcgttatactaaagaacttgaggatgttaaaactaaagtttatacgagagatttatttggccgtgactaaacaacaattttggaggaaaaattggaacgaaaaaaaaagaaaaaaaagaatatttgggttataattatacctatcttaatttttattacccttataggagcaggggcttatgccttaagagattcacttatttctactgatcatacgaaaacaaatagttcggatcaaccgaccaaaacttcggcctctaatggttatgtagagaaaaaaggtaaagaagctgctgtgggtagtatagcacttgtagatgatgttggtataccagaatggattaaggttccctcaaaggcaaatctagataaatttactgatttatctacgaataatatcactatttatcgaattaataatccggaagtcttaaaaacagttaccaatcgtacagatcaacggatgaaaatgtcagaagttatagctaagtatcctaatgctttgattatgaatgcttccgcttttgatatgcagacaggacaagtagttggatttcaaatgaataatggaaagttaattcaagactggaatccaggtacaacgactcaatatgcttttgttattaacaaagatggttcatgcaaaatttatgattcaagtacacctgcttcaactattattaaaaacggagggcaacaagcctatgattttggtacggcaattatccgtgatggtaaaattcaaccaagtgatggctcagtagattggaagatccatatttttattgcgaatgataaagataataatctctatgctattttgagtgatacaaatgcaggttatgataatataatgaagtcagtgtcaaatttgaagctccaaaatatgctgttacttgatagtggtggctcaagtcaactatctgtcaatggtaaaacgattgttgctagtcaagatgatcgagccgtgccggattatattgtgatgaaataaaaataaaagaacctcttggttcttttattttagagatttttcaaaaagggttttgactgagtctaattctgtttgagaaacgaccttagctccattttcatctgttgtatgtagattaagcttgccggtattctttagagccttattgtagctcataacgatcgttttagcatcattgaaacttatattggttttaacagtgtttgaaaaagcatagagaatttcgcgatagtaattgaaactttcaagttttttcatatgagcaactttttgaatatttccgtagagttccattgagacattttgaatccgagtgattgaagcatccaaatcagtatcgtcaatttgtgtcatataggcttggacttgatcagcagtttgtaaattaacagttccttgtttaaactcataaccttcagcattgaatgcctttggattttgcatggtgattccaccagtagcctgtacaagtgatcccattttattaacatcaatctgaattactttgttaatggacacattcaataggtctttaaccatctggaaaattccatcatctccattcgtattgtaaacttcagtgattgttttttgattaggcattgtcgcaaaaactgggaagttcatgaaagtagtttgatttgtctttacattcgttgaagctaaaacagtagcataagctgtatttttagaattatttttaccagttgcaatgataagtgtggtgaatgttttagatttttttaagtcaatacttgttgttttagggaaattttcatatgatgttgaaaaggttgattcaacatttctataagctacgtaggctatagaagcaacagcgataattactaatacaaaaataattgaaataacttttagtactgtgtgttttttcttacgataatgacgcctctttttttgattcat

SEQ ID NO: 2 - DNA, 318 bp, Lactococcus lactis subsp. lactis
atgaatgatttgttttaccatcgtctaaaggaactagttgaatcaagtggtaaatctgcaaatcaaatagagagggaattgggttaccctagaaattctttgaataattataagttaggaggagaaccctctgggacaagattaataggactatcggagtattttagtgtgtctccaaaatatctgatgggtataattgatgagcctaatgatagttctgcaattaatctttttaaaagtctaactcaagaagagaaaaaagaaatgtgtataatttgtcaaaaatggctttttttagaatatcaaatagaattataa

SEQ ID NO: 3 - DNA, 768 bp, Lactococcus lactis subsp. lactis
atgatgaaaaaaggaatttttgtaattactatagtgatatctatagcattgataattggaggtttttatagttataattctaggataaataatctttcaaaaactaataacggaaaagaagttgtaaaaaatagcagtgaaaaaaatcagatagaacttacctataaaaagtattataaaaatttaccaaaatcagttcaaaataaaatagatgatatttcatccaaaaataaagaagttactttaacttgtatttggcaatctgattcagttatttctgaacaatttcaacaaaacttacaaaaatattatggaaataagttttggaacatcaaaaatatcacttacaatggcgaaactagtgaacaattattggctgaaaaagttgaaaatcaagtattagccactaatcctgatgttgttttatatgaagctccactttttaatgataaccaaaacattgaagcaacagcctcactgactagtaatgagcaacttataacaaatttggctagtgcaggagcggaggtaatagttcaaccctctccaccgatctatggtggtgttgtgtaccccgtacaagaagaacaatttaaacaatctttatctacaaagtatccctatatagactactgggctagttacccagacaaaaattctgatgaaatgaaggggctgttttctgataatggagtatatagaacattaaatgcttcggggaataaggtttggctagattatattactaaatattttacagcaaactaa

SEQ ID NO: 4 - DNA, 780 bp, Lactococcus lactis subsp. lactis
atgcaggaaacacaggaacaaacgattgatttaagagggatttttaaaattattcgcaaaaggttaggtttaatattatttagtgctttaatagtcacaatattagggagcatctacacattttttatagcctccccagtttacacagcctcaactcaacttgtcgttaaactaccaaattcggataattcagcagcctacgctggacaagtgaccgggaatattcaaatggcgaacacaattaaccaagttattgttagtccagtcattttagataaagttcaaagtaatttaaatctatctgatgactctttccaaaaacaagttacagcagcaaatcaaacaaattcacaagtcattacgcttactgttaaatattctaatccttacgttgctcaaaagattgcagacgagactgctaaaatatttagttcagacgcagcgaaactattgaatgttactaacgttaatattctatccaaagcaaaagctcaaacaacacccattagtcctaaacctaaattgtatttagcaatatctgttatagccggattagttttaggtttagccattgctttattgaaggaattgtttgataacaaaattaataaagaagaagatattgaagctctgggactcacggttcttggtgtaacaacctatgctcaaatgagtgattttaataagaatacgaataaaaatggcacgcaatcgggaactaagtcaagtccgcctagcgaccatgaagtaaatagatcatcaaaaaggaataaaagatag

SEQ ID NO: 5 - DNA, 696 bp, Lactococcus lactis subsp. lactis
atggctaaaaataaaagaagcatagacaacaatcgttatattattaccagtgtcaatcctcaatcacctatttccgaacaatatcgtacgattcgtacgaccattgattttaaaatggcggatcaagggattaaaagttttctagtaacatcttcagaagcagctgcaggtaaatcaaccgtaagtgctaatctagctgttgcttttgcacaacaaggtaaaaaagtacttttaattgatggcgatcttcgtaaaccgactgttaacattacttttaaagtacaaaatagagtaggattaaccaatattttaatgcatcaatcttcgattgaagatgccatacaagggacaagactttctgaaaatcttacaataattacctctggtccaattccacctaatccatcggaattattagcatctagtgcaatgaagaatttgattgactctgtgtccgattcctttgatattgttttgattgatactccacctctctctgcagttactgatgctcaaattttgagtatttatgtaggaggagtggttcttgttgtacgtgcctatgaaacaaaaaaagagagtttagcaaaaacaaaaaaaatactggaacaagttaatgtaaatatattaggagttgttttgcatggggtagactcttctgagtcaccgtcgtattactactacggagtagagtaa

SEQ ID NO: 6 - DNA, 765 bp, Lactococcus lactis subsp. lactis
atgattgatattcattgccatattttaccggggatagatgatggagctaaaacttctggtgatactctgacaatgctgaaatcagcaattgatgaagggataacagctatcactgcaactcctcatcataatcctcaatttaataatgaatcaccgcttattttgaaaaaagttaaggaagttcaaaatatcattgacgaacatcaattaccaattgaagttttacccggacaagaggtgagaatatatggtgatttattaaaagaattttctgaagggaagttactgacagcagcgggcacttcaagttatatactgattgaatttccatcaaatcatgtgccagcttatgctaaagaacttttttataatattcaattggagggacttcaacctattttggttcaccctgagcgtaatagtgcaatcattgagaaccctgatatattatttgattttattgaacaaggagtactaagtcagataacagcttcaagtgtcactggtcattttggtaaaaaaatacaaaagctgtcatttaaaatgatagaaaaccatctgacgcattttgttgcatcagatgcgcataatgtgacgtcacgtgcatttaagatgaaggaagcatttgaaatgattgaagatagttatggttctggtgtatcacgaaggtttaaagataatgcagagtcagtgattttaaacgaaagtttttatcaagaaaaaccaacaaagatcaaaacaaaaaaatttttaggattattttaa

SEQ ID NO: 7 - DNA, 687 bp, Lactococcus lactis subsp. lactis
atggaagtttttgaggatgcctcatcacctgaatcggaagaacacaaattagtagtattaaaaaatttttcttatggagagctgattataaaaagagcaattgatatcctaggaggattagcgggttcagttttatttcttatcgcggctgcattgctttatgtcccttacaaaatgagctcggaaaaagatcaagggccaatgttctataaacaaaaacgggttggaaaaaacggtaaaattttttatattttgaaatttagaacaatgataattaatgctgagcagtatctagagctacatccagaagttaaagccgcctatcatgccaatggtaataaactagaaaatgatccccgtgtgacgaagattggttcatttattagacaatactcagttgatgaattaccacaatttatcaatgtccttaaaggagatatggcattagtcggtccaaggccaattcaacattttgaagcgaaagaatttggggagcgcctcccttatttactgatatgtaaacctggaattactggttattggacaacacatggtcgcagtaaagctccttttcctcaacgagcagatttagaactctattatctccaatatcacagcaccaagaatgatgtcaagcttcttatgcttacaattgcacaaattattcacggatcggacgcatattaa

SEQ ID NO: 8 - DNA, 1122 bp, Lactococcus lactis subsp. lactis
atgaaaaaaaagaaattattactaataagtcaaagcggaagaggtggagtaaggaaacatctttgtgatttacttacttctcttgattataaaaaatttgagatttggattgcctataatgatgatgaggtcgatgagatttttaaatatacgttggaaagtttaaggggaaaagttaaaccaatcattataaaagaaatggttagagaacttaatcctaaacaagattggattgcatttaagaaaattcgtaggtcaataaaagagataaaaccagatattgttcattgccatagttcgaaagcgggaatattagggcgagcagctgcaaaaatagtgggtataaaacaaatatattacacacctcacgcttactcttttctcgctacagaattttcagtaaaaaagaaaagattattcattaatctagaacgtttttttagtcattatgctacaactttaacatttaccgtgtcagaaggtgaaaaagaagcagcactaaaaaacaaagttgatagcaatgagaaatttaaagtaatttataatggattgaaagatataaaaatcttatctaaaatagaagccagggaaaaacttggattaccacaagataaatttatttttggtaatattgctcgaatttgtgaacaaaaaaatccaatttattttatagaagttgctcaaaaaaatcctgattattattttgtttggattggtgatggtgaacttcgtgagaaagtcaaacaagaaattctctatagaaacctgaaaaatatttgtttcttaggaaatagaaatgatgcaggaataatggtcgcggcattcgatgtgtttatatctacttctaaatatgaaggactgccctattcacctattgaagctctccgagctggagtgcctgttttgttaagtgatgttgttggtaataatgaagttgtcttaagccatagaaatggggaagtttttgatttaaattcgtctaattggaataaaagacttgatgaatttagaaagtggcaaaagaagaaaacgagtatagagatcagacaaacgtttcttaatcacttctcattggataaatcgataaaagaactaactaagatatatttgaataatgagtaa

SEQ ID NO: 9 - DNA, 1104 bp, Lactococcus lactis subsp. lactis
atgcttatttattttcttttatttcctataattattttattatatatttttacaaacaacggactattaaagagtaaaaaaatatttataggactttcattctccatactagggattatttcgtctatacgttctcctcaagtaggaaccgatacatcaacttaccaaacacttttcttctatcaaatacatggaataaaaatattcaattcaaacaatccggagttaagcagcaaagctccactttatggtgtatatagtcgtattgtaagtatgatttcagtaaatttacagaccattactatagctaattcattgctgatagcattcttatttggaatttttatttatagattgaaaattaatccgctatattcaactttattatttattagtattggatttttcacaagttctcttaatacatctcgacagtttatcgctatcggtttagtatgcaatgctctgctatttctatttgataaaaaggcatttatatattttgctttaatcacattagcaatatctattcatacgctagcaatagttggattgatattttatccgatttataagattaaatggacagcagtaaaaatatcctgttttctaattgtgttgacaatgacaagctttttccttgagtctgtttcgaaaatttttattcaatttttccccaattacgctttttacttacaaaatcccgtgacattctttggtgcttctagccgtataataatgattttagatattggactaattttaattattttattattttatgcgttgactaaatactatcatattaagtgtagtcaagaagaagtttctttgcttatcattttcttaattggaccattttttgaaatacttgtatttcacaatcagagtatattacttttgactcaacgatttctaacttttttttctattttaagtattgctgtaattccaggaatgtgtgctaaagtttcaaaaaaattcaataacccagaaaatgtgagttttgctttttttagtgttatatttattttcacattatttactttttctgtagaaattcaaaaatattggggagttattccctatattacttttatgtaa

SEQ ID NO: 10 - DNA, 876 bp, Lactococcus lactis subsp. lactis
atgctaatttctgtaataattccaatgtataatagaaaatttacaataaagagagctatgaacagtgtactttctcaagtaccaaataaaaaggagtttcaaattgaattaattgttgttgatgactgctccactgacaatagtgttgaggttgctagagaaataaaggatgaacgggtaaaaattgtcaaacttgataaaaactcgggtgctaatgttgcgagaaattatggaattaatttagcaaatggtgagataatcgcttttaatgattcagatgatgaatggcttcctgaaaaactttctaagcaacttgaagtacttcaagaaaaaaatatagattttttgtgctgtaatatggaaacggatgtttacagtggaaaaatgaaaatgcttacgcctagaccgtcaggttttgttccaattgaagaattgcttggaaaaaattatatagtaagtactcagaatttgattggaaaagctgatatgtttaaatctaatcaattcagtcatgaaatctctcgttttcaagactgggagcttattctacggcttttgattaaggggtataggctttattttatggaagaagtattagtgagacagtatattcaaccaaatagtttatccaaaaatttaaaaaatggtgttttgtctctccgatatatgcttgaggaattcaaagaagagtatgcacagcatcctttacaaaaggcagaggtaatattaactgttggtagccatttacacaatatgaattatcgatgtgctcaattttattttaaatctttgaagttaagatttagcatgactgtattggcaaaagcactttttatgttttttacggacttatcaagaaagaaggaaagcgaatga

SEQ ID NO: 11 - DNA, 897 bp, Lactococcus lactis subsp. lactis
atgacagagaggattacagtgattctttccgcatataacggtgagaaatatattcaaagtcaaatagacagtatacttaatcaaacatatgataattttattttatatattagagatgatggatcaactgacggaactcgaaaaattctgaagcaatattctgaaaaagattcacgagtgaaagttcaatatggtgaaaacataggctatgtaaaaagtttttttaaaatgctttctgaagtcaattcggaatatatagcattttctgatcaagatgatatttggctgcctgaaaagttatcagtcgctcaagcagctttatcacagaaaaataagagcgttcctctcatgtgggcctcaaatatatatatatgtgatgaaaaaatgaatgtaatttcgattggtgcaaggaagagaatgagtaatttctcaaattctctttttatgtgtaatactcaaggaatgacaatgataattaataataaagctagagaaaaggttgtttctaatctaccaaaacaaaatatcatgtaccacgattggtggatttatcgcgttgttagtgctttcggagaagttatatttgattcagatccatatgtaaagtatagaagacatgataaaaatgaatctgatatttcatataattttgtgaataaagtcactaatatgatgaaccgcttaataaatagcgatatgtatatacgtacgaagaaagagacacaagaatttaaaataatttttgattcacaactttcacaatcaaatagagatgtattaagtttatttgcctcaccaaaaagaaaaattcaaaaagtcttctactcaggtagattcaaaaattccgtattagatgaactagtacttcgcttattttttcttttagacattttataa

SEQ ID NO: 12 - DNA, 1422 bp, Lactococcus lactis subsp. lactis
atgaataataaattaagagaaggttttacttttacagcaattggtacatatagtaattttttaattcaaattattgtacaagcaattttaagtcgattattatcgccaagagagtatggaataattgctatcatgcaagtttttatagttttttttgcaatgctggtggaagcaggaatgggacctgctatcatacaaaataaaaagttaacaaacagagacaatatgaatttatttaacttttcagctattttttctattatatttgcgattatatttggttttttaggattattacttacaaagatatatatgaatccagcatacacttacttaacttggattcagtctatttcaatattatttattgggttaaatattgttccgactgcactccttaataaaagaaaacaattcaaagctgtaaattttagtacagtagtaggggggatactatcgggagtagtcggagttacaatggctttcctgggatttggtatttattcactaattgcaagtgccattacaacggcatttgtaagtttttgcttaaacaggtattttgctaatatttggtttactaaaaattggaataaatcttctttgatttctatttggactgtttcgcggaatcagtttggaacaaattttataaattatttttcgaataattcagacaatattttagtaggaaaatttatgggagatacagcactagctaattacaataagtcttatcaactgttaacaatccctaccactttattgttgaatatagttaatccagttttacaaccaattctctcagattatcaagatgatgttgtaactataagaaaaacatactataatattgttcacttattggctctcatcgggattcctacatcaatttttcttagtatgtctgcaaaacaaattatttttttcttttttggaagtcagtgggaagaagcagtagttcccttctcttacttagcagttattgtatggtgtcaaatgacaacatattcaaatggagcaatctggcagtccagaaataaaacaaattattttcttttttcaagtgttatcaatacttttattataattttttctatcataataggtatcataataggaaatataaatgcggttgctttatttgttgcaataggaaattttataagttttttttggaaattctactatattactaaaaatgcattagaagattctataagaaatctactaaagattttcatccatcctatttttttaggattcatcacatttattgggattagattagagattttaattgatcctagaaataatttttttagtctacttctaagaagcttagtatttttttctattctaattacctatattatgtttacatctgaaaagaaaataattgaagaaatttttgataaatag

SEQ ID NO: 13 - DNA, 1167 bp, Lactococcus lactis subsp. lactis
atgaaaatagcagttgttgggacaggctatgtcggtttgtctatttcagtgcttctagcacaacatcatgaagttgttgctttggatattgttgaggcgaaagtagatttgattaactctaaaaaatcgcctattgttgataaggagattgagggatttttagcaagtaaagaattaaatttacttgcgacgacggatacggctcaagcgctaaatagagctgactttgtggtcattgcaacacctaccaattatgatgatgtcaagaattattttaatacggattctgtagaagcagtaattgaagaagtttggaaatttagcccaaatgctatgattgttataaaatcaactattccagttggttttgtggaaaaaatgcgtgctaaatatgatattgataacattatcttttctccagaatttttacgagaaggtcgagcattgtatgacaatcttcatccatctcgcattgttgtgggggaacaatctgagcgtgcctctcaatttgctgagcttttaatagagggagctattgataaagatatcccagttctttttacaaaccctactgaagcagaagcgattaagctattttcaaatacatatttagctttacgcgtggcttattttaatgaattagatacttatgctgaagttcgtggtttagatacaaaacaaatcattgatggcgttggattagatccacgaattggaacacactacaataatccttcatttggttatggagggtattgcctaccgaaagataccaaacagcttttagctaactacgaccaagttcctgaaaaattaattgaggctgttgttgaatcaaatagtacaagaaaagatcatattgcagatatgatcattaaacgttctcctaaagtggtgggtatctaccgcttgactatgaagtcaaattctgataattttagatcaagttcaattcaaggaattatgaaacgaattaagggcaagggaattgaagtagttgtctatgagccaacactaaatgatactcatttctacaattctcgggtagttcataatttggatgagtttaaaacgatttctgatgtgattgtttcaaatcgttatactaaagaacttgaggatgttaaaactaaagtttatacgagagatttatttggccgtgactaa

SEQ ID NO: 14 - DNA, 903 bp, Lactococcus lactis subsp. lactis
ttggaacgaaaaaaaaagaaaaaaaagaatatttgggttataattatacctatcttaatttttattacccttataggagcaggggcttatgccttaagagattcacttatttctactgatcatacgaaaacaaatagttcggatcaaccgaccaaaacttcggcctctaatggttatgtagagaaaaaaggtaaagaagctgctgtgggtagtatagcacttgtagatgatgttggtataccagaatggattaaggttccctcaaaggcaaatctagataaatttactgatttatctacgaataatatcactatttatcgaattaataatccggaagtcttaaaaacagttaccaatcgtacagatcaacggatgaaaatgtcagaagttatagctaagtatcctaatgctttgattatgaatgcttccgcttttgatatgcagacaggacaagtagttggatttcaaatgaataatggaaagttaattcaagactggaatccaggtacaacgactcaatatgcttttgttattaacaaagatggttcatgcaaaatttatgattcaagtacacctgcttcaactattattaaaaacggagggcaacaagcctatgattttggtacggcaattatccgtgatggtaaaattcaaccaagtgatggctcagtagattggaagatccatatttttattgcgaatgataaagataataatctctatgctattttgagtgatacaaatgcaggttatgataatataatgaagtcagtgtcaaatttgaagctccaaaatatgctgttacttgatagtggtggctcaagtcaactatctgtcaatggtaaaacgattgttgctagtcaagatgatcgagccgtgccggattatattgtgatgaaataa

SEQ ID NO: 15 - DNA, 903 bp, Lactococcus lactis subsp. lactis
atgaatcaaaaaaagaggcgtcattatcgtaagaaaaaacacacagtactaaaagttatttcaattatttttgtattagtaattatcgctgttgcttctatagcctacgtagcttatagaaatgttgaatcaaccttttcaacatcatatgaaaatttccctaaaacaacaagtattgacttaaaaaaatctaaaacattcaccacacttatcattgcaactggtaaaaataattctaaaaatacagcttatgctactgttttagcttcaacgaatgtaaagacaaatcaaactactttcatgaacttcccagtttttgcgacaatgcctaatcaaaaaacaatcactgaagtttacaatacgaatggagatgatggaattttccagatggttaaagacctattgaatgtgtccattaacaaagtaattcagattgatgttaataaaatgggatcacttgtacaggctactggtggaatcaccatgcaaaatccaaaggcattcaatgctgaaggttatgagtttaaacaaggaactgttaatttacaaactgctgatcaagtccaagcctatatgacacaaattgacgatactgatttggatgcttcaatcactcggattcaaaatgtctcaatggaactctacggaaatattcaaaaagttgctcatatgaaaaaacttgaaagtttcaattactatcgcgaaattctctatgctttttcaaacactgttaaaaccaatataagtttcaatgatgctaaaacgatcgttatgagctacaataaggctctaaagaataccggcaagcttaatctacatacaacagatgaaaatggagctaaggtcgtttctcaaacagaattagactcagtcaaaaccctttttgaaaaatctctaaaataa

SEQ ID NO: 16 - DNA, 7097 bp, Lactococcus lactis subsp. lactis
aaaacaatgaaaaaaaagaaattattactaataagtcaaagcggaagaggtggagtaaggaaacatctttgtgatttacttacttctcttgattataaaaaatttgagatttggattgcctataatgatgatgaggtcgatgagatttttaaatatacgttggaaagtttaaggggaaaagttaaaccaatcattataaaagaaatggttagagaacttaatcctaaacaagattggattgcatttaagaaaattcgtaggtcaataaaagagataaaaccagatattgttcattgccatagttcgaaagcgggaatattagggcgagcagctgcaaaaatagtgggtataaaacaaatatattacacacctcacgcttactcttttctcgctacagaattttcagtaaaaaagaaaagattattcattaatctagaacgtttttttagtcattatgctacaactttaacatttaccgtgtcagaaggtgaaaaagaagcagcactaaaaaacaaagttgatagcaatgagaaatttaaagtaatttataatggattgaaagatataaaaatcttatctaaaatagaagccagggaaaaacttggattaccacaagataaatttatttttggtaatattgctcgaatttgtgaacaaaaaaatccaatttattttatagaagttgctcaaaaaaatcctgattattattttgtttggattggtgatggtgaacttcgtgagaaagtcaaacaagaaattctctatagaaacctgaaaaatatttgtttcttaggaaatagaaatgatgcaggaataatggtcgcggcattcgatgtgtttatatctacttctaaatatgaaggactgccctattcacctattgaagctctccgagctggagtgcctgttttgttaagtgatgttgttggtaataatgaagttgtcttaagccatagaaatggggaagtttttgatttaaattcgtctaattggaataaaagacttgatgaatttagaaagtggcaaaagaagaaaacgagtatagagatcagacaaacgtttcttaatcacttctcattggataaatcgataaaagaactaactaagatatatttgaataatgagtaataggcaacagttacatagctattttcatccaacaagtgattctatggctttcctatgatcaacaaatttagtagttatgttttattgtagcctaatattccaaaacaatttaaaacattaaaattcaagtaactttttagttaattaaattcggataggcttaataaaattgtggattaaattaacttatatgcagattctactgagattagggtcatgatcgcttgtattaattatttcacacataaccaggagtaagatttatgcttatttattttcttttatttcctataattattttattatatatttttacaaacaacggactattaaagagtaaaaaaatatttataggactttcattctccatactagggattatttcgtctatacgttctcctcaagtaggaaccgatacatcaacttaccaaacacttttcttctatcaaatacatggaataaaaatattcaattcaaacaatccggagttaagcagcaaagctccactttatggtgtatatagtcgtattgtaagtatgatttcagtaaatttacagaccattactatagctaattcattgctgatagcattcttatttggaatttttatttatagattgaaaattaatccgctatattcaactttattatttattagtattggatttttcacaagttctcttaatacatctcgacagtttatcgctatcggtttagtatgcaatgctctgctatttctatttgataaaaaggcatttatatattttgctttaatcacattagcaatatctattcatacgctagcaatagttggattgatattttatccgatttataagattaaatggacagcagtaaaaatatcctgttttctaattgtgttgacaatgacaagctttttccttgagtctgtttcgaaaatttttattcaatttttccccaattacgctttttacttacaaaatcccgtgacattctttggtgcttctagccgtataataatgattttagatattggactaattttaattattttattattttatgcgttgactaaatactatcatattaagtgtagtcaagaagaagtttctttgcttatcattttcttaattggaccattttttgaaatacttgtatttcacaatcagagtatattacttttgactcaacgatttctaacttttttttctattttaagtattgctgtaattccaggaatgtgtgctaaagtttcaaaaaaattcaataacccagaaaatgtgagttttgctttttttagtgttatatttattttcacattatttactttttctgtagaaattcaaaaatattggggagttattccctatattacttttatgtaattagaaaggtttatttaaatatgctaatttctgtaataattccaatgtataatagaaaatttacaataaagagagctatgaacagtgtactttctcaagtaccaaataaaaaggagtttcaaattgaattaattgttgttgatgactgctccactgacaatagtgttgaggttgctagagaaataaaggatgaacgggtaaaaattgtcaaacttgataaaaactcgggtgctaatgttgcgagaaattatggaattaatttagcaaatggtgagataatcgcttttaatgattcagatgatgaatggcttcctgaaaaactttctaagcaacttgaagtacttcaagaaaaaaatatagattttttgtgctgtaatatggaaacggatgtttacagtggaaaaatgaaaatgcttacgcctagaccgtcaggttttgttccaattgaagaattgcttggaaaaaattatatagtaagtactcagaatttgattggaaaagctgatatgtttaaatctaatcaattcagtcatgaaatctctcgttttcaagactgggagcttattctacggcttttgattaaggggtataggctttattttatggaagaagtattagtgagacagtatattcaaccaaatagtttatccaaaaatttaaaaaatggtgttttgtctctccgatatatgcttgaggaattcaaagaagagtatgcacagcatcctttacaaaaggcagaggtaatattaactgttggtagccatttacacaatatgaattatcgatgtgctcaattttattttaaatctttgaagttaagatttagcatgactgtattggcaaaagcactttttatgttttttacggacttatcaagaaagaaggaaagcgaatgacagagaggattacagtgattctttccgcatataacggtgagaaatatattcaaagtcaaatagacagtatacttaatcaaacatatgataattttattttatatattagagatgatggatcaactgacggaactcgaaaaattctgaagcaatattctgaaaaagattcacgagtgaaagttcaatatggtgaaaacataggctatgtaaaaagtttttttaaaatgctttctgaagtcaattcggaatatatagcattttctgatcaagatgatatttggctgcctgaaaagttatcagtcgctcaagcagctttatcacagaaaaataagagcgttcctctcatgtgggcctcaaatatatatatatgtgatgaaaaaatgaatgtaatttcgattggtgcaaggaagagaatgagtaatttctcaaattctctttttatgtgtaatactcaaggaatgacaatgataattaataataaagctagagaaaaggttgtttctaatctaccaaaacaaaatatcatgtaccacgattggtggatttatcgcgttgttagtgctttcggagaagttatatttgattcagatccatatgtaaagtatagaagacatgataaaaatgaatctgatatttcatataattttgtgaataaagtcactaatatgatgaaccgcttaataaatagcgatatgtatatacgtacgaagaaagagacacaagaatttaaaataatttttgattcacaactttcacaatcaaatagagatgtattaagtttatttgcctcaccaaaaagaaaaattcaaaaagtcttctactcaggtagattcaaaaattccgtattagatgaactagtacttcgcttattttttcttttagacattttataattaaaaaattttttaatagttatacattataagataagttgtttgtatagtactttaatggtattaaattatagaggtaagctattagacgagaatttttttattttacaacttggaaaacagactctaacaaggggaaatgagaaataaatgaataataaattaagagaaggttttacttttacagcaattggtacatatagtaattttttaattcaaattattgtacaagcaattttaagtcgattattatcgccaagagagtatggaataattgctatcatgcaagtttttatagttttttttgcaatgctggtggaagcaggaatgggacctgctatcatacaaaataaaaagttaacaaacagagacaatatgaatttatttaacttttcagctattttttctattatatttgcgattatatttggttttttaggattattacttacaaagatatatatgaatccagcatacacttacttaacttggattcagtctatttcaatattatttattgggttaaatattgttccgactgcactccttaataaaagaaaacaattcaaagctgtaaattttagtacagtagtaggggggatactatcgggagtagtcggagttacaatggctttcctgggatttggtatttattcactaattgcaagtgccattacaacggcatttgtaagtttttgcttaaacaggtattttgctaatatttggtttactaaaaattggaataaatcttctttgatttctatttggactgtttcgcggaatcagtttggaacaaattttataaattatttttcgaataattcagacaatattttagtaggaaaatttatgggagatacagcactagctaattacaataagtcttatcaactgttaacaatccctaccactttattgttgaatatagttaatccagttttacaaccaattctctcagattatcaagatgatgttgtaactataagaaaaacatactataatattgttcacttattggctctcatcgggattcctacatcaatttttcttagtatgtctgcaaaacaaattatttttttcttttttggaagtcagtgggaagaagcagtagttcccttctcttacttagcagttattgtatggtgtcaaatgacaacatattcaaatggagcaatctggcagtccagaaataaaacaaattattttcttttttcaagtgttatcaatacttttattataattttttctatcataataggtatcataataggaaatataaatgcggttgctttatttgttgcaataggaaattttataagttttttttggaaattctactatattactaaaaatgcattagaagattctataagaaatctactaaagattttcatccatcctatttttttaggattcatcacatttattgggattagattagagattttaattgatcctagaaataatttttttagtctacttctaagaagcttagtatttttttctattctaattacctatattatgtttacatctgaaaagaaaataattgaagaaatttttgataaatagtcaatgcatctataagatactaaaggattccaaaaatatataaggagaaaaacatgaaaatagcagttgttgggacaggctatgtcggtttgtctatttcagtgcttctagcacaacatcatgaagttgttgctttggatattgttgaggcgaaagtagatttgattaactctaaaaaatcgcctattgttgataaggagattgagggatttttagcaagtaaagaattaaatttacttgcgacgacggatacggctcaagcgctaaatagagctgactttgtggtcattgcaacacctaccaattatgatgatgtcaagaattattttaatacggattctgtagaagcagtaattgaagaagtttggaaatttagcccaaatgctatgattgttataaaatcaactattccagttggttttgtggaaaaaatgcgtgctaaatatgatattgataacattatcttttctccagaatttttacgagaaggtcgagcattgtatgacaatcttcatccatctcgcattgttgtgggggaacaatctgagcgtgcctctcaatttgctgagcttttaatagagggagctattgataaagatatcccagttctttttacaaaccctactgaagcagaagcgattaagctattttcaaatacatatttagctttacgcgtggcttattttaatgaattagatacttatgctgaagttcgtggtttagatacaaaacaaatcattgatggcgttggattagatccacgaattggaacacactacaataatccttcatttggttatggagggtattgcctaccgaaagataccaaacagcttttagctaactacgaccaagttcctgaaaaattaattgaggctgttgttgaatcaaatagtacaagaaaagatcatattgcagatatgatcattaaacgttctcctaaagtggtgggtatctaccgcttgactatgaagtcaaattctgataattttagatcaagttcaattcaaggaattatgaaacgaattaagggcaagggaattgaagtagttgtctatgagccaacactaaatgatactcatttctacaattctcgggtagttcataatttggatgagtttaaaacgatttctgatgtgattgtttcaaatcgttatactaaagaacttgaggatgttaaaactaaagtttatacgagagatttatttggccgtgactaaacaacaattttggaggaaaaa

SEQ ID NO: 17 - protein, 105 aa, Lactococcus lactis subsp. lactis
MNDLFYHRLKELVESSGKSANQIERELGYPRNSLNNYKLGGEPSGTRLIGLSEYFSVSPKYLMGIIDEPNDSSAINLFKSLTQEEKKEMCIICQKWLFLEYQIEL

SEQ ID NO: 18 - protein, 255 aa, Lactococcus lactis subsp. lactis
MMKKGIFVITIVISIALIIGGFYSYNSRINNLSKTNNGKEVVKNSSEKNQIELTYKKYYKNLPKSVQNKIDDISSKNKEVTLTCIWQSDSVISEQFQQNLQKYYGNKFWNIKNITYNGETSEQLLAEKVENQVLATNPDVVLYEAPLFNDNQNIEATASLTSNEQLITNLASAGAEVIVQPSPPIYGGVVYPVQEEQFKQSLSTKYPYIDYWASYPDKNSDEMKGLFSDNGVYRTLNASGNKVWLDYITKYFTAN

SEQ ID NO: 19 - protein, 259 aa, Lactococcus lactis subsp. lactis
MQETQEQTIDLRGIFKIIRKRLGLILFSALIVTILGSIYTFFIASPVYTASTQLVVKLPNSDNSAAYAGQVTGNIQMANTINQVIVSPVILDKVQSNLNLSDDSFQKQVTAANQTNSQVITLTVKYSNPYVAQKIADETAKIFSSDAAKLLNVTNVNILSKAKAQTTPISPKPKLYLAISVIAGLVLGLAIALLKELFDNKINKEEDIEALGLTVLGVTTYAQMSDFNKNTNKNGTQSGTKSSPPSDHEVNRSSKRNKR

SEQ ID NO: 20 - protein, 231 aa, Lactococcus lactis subsp. lactis
MAKNKRSIDNNRYIITSVNPQSPISEQYRTIRTTIDFKMADQGIKSFLVTSSEAAAGKSTVSANLAVAFAQQGKKVLLIDGDLRKPTVNITFKVQNRVGLTNILMHQSSIEDAIQGTRLSENLTIITSGPIPPNPSELLASSAMKNLIDSVSDSFDIVLIDTPPLSAVTDAQILSIYVGGVVLVVRAYETKKESLAKTKKILEQVNVNILGVVLHGVDSSESPSYYYYGVE

SEQ ID NO: 21 - protein, 254 aa, Lactococcus lactis subsp. lactis
MIDIHCHILPGIDDGAKTSGDTLTMLKSAIDEGITAITATPHHNPQFNNESPLILKKVKEVQNIIDEHQLPIEVLPGQEVRIYGDLLKEFSEGKLLTAAGTSSYILIEFPSNHVPAYAKELFYNIQLEGLQPILVHPERNSAIIENPDILFDFIEQGVLSQITASSVTGHFGKKIQKLSFKMIENHLTHFVASDAHNVTSRAFKMKEAFEMIEDSYGSGVSRRFKDNAESVILNESFYQEKPTKIKTKKFLGLF

SEQ ID NO: 22 - protein, 228 aa, Lactococcus lactis subsp. lactis
MEVFEDASSPESEEHKLVVLKNFSYGELIIKRAIDILGGLAGSVLFLIAAALLYVPYKMSSEKDQGPMFYKQKRVGKNGKIFYILKFRTMIINAEQYLELHPEVKAAYHANGNKLENDPRVTKIGSFIRQYSVDELPQFINVLKGDMALVGPRPIQHFEAKEFGERLPYLLICKPGITGYWTTHGRSKAPFPQRADLELYYLQYHSTKNDVKLLMLTIAQIIHGSDAY

SEQ ID NO: 23 - protein, 373 aa, Lactococcus lactis subsp. lactis
MKKKKLLLISQSGRGGVRKHLCDLLTSLDYKKFEIWIAYNDDEVDEIFKYTLESLRGKVKPIIIKEMVRELNPKQDWIAFKKIRRSIKEIKPDIVHCHSSKAGILGRAAAKIVGIKQIYYTPHAYSFLATEFSVKKKRLFINLERFFSHYATTLTFTVSEGEKEAALKNKVDSNEKFKVIYNGLKDIKILSKIEAREKLGLPQDKFIFGNIARICEQKNPIYFIEVAQKNPDYYFVWIGDGELREKVKQEILYRNLKNICFLGNRNDAGIMVAAFDVFISTSKYEGLPYSPIEALRAGVPVLLSDVVGNNEVVLSHRNGEVFDLNSSNWNKRLDEFRKWQKKKTSIEIRQTFLNHFSLDKSIKELTKIYLNNE

SEQ ID NO: 24 - protein, 367 aa, Lactococcus lactis subsp. lactis
MLIYFLLFPIIILLYIFTNNGLLKSKKIFIGLSFSILGIISSIRSPQVGTDTSTYQTLFFYQIHGIKIFNSNNPELSSKAPLYGVYSRIVSMISVNLQTITIANSLLIAFLFGIFIYRLKINPLYSTLLFISIGFFTSSLNTSRQFIAIGLVCNALLFLFDKKAFIYFALITLAISIHTLAIVGLIFYPIYKIKWTAVKISCFLIVLTMTSFFLESVSKIFIQFFPNYAFYLQNPVTFFGASSRIIMILDIGLILIILLFYALTKYYHIKCSQEEVSLLIIFLIGPFFEILVFHNQSILLLTQRFLTFFSILSIAVIPGMCAKVSKKFNNPENVSFAFFSVIFIFTLFTFSVEIQKYWGVIPYITFM

SEQ ID NO: 25 - protein, 291 aa, Lactococcus lactis subsp. lactis
MLISVIIPMYNRKFTIKRAMNSVLSQVPNKKEFQIELIVVDDCSTDNSVEVAREIKDERVKIVKLDKNSGANVARNYGINLANGEIIAFNDSDDEWLPEKLSKQLEVLQEKNIDFLCCNMETDVYSGKMKMLTPRPSGFVPIEELLGKNYIVSTQNLIGKADMFKSNQFSHEISRFQDWELILRLLIKGYRLYFMEEVLVRQYIQPNSLSKNLKNGVLSLRYMLEEFKEEYAQHPLQKAEVILTVGSHLHNMNYRCAQFYFKSLKLRFSMTVLAKALFMFFTDLSRKKESE

SEQ ID NO: 26 - protein, 298 aa, Lactococcus lactis subsp. lactis
MTERITVILSAYNGEKYIQSQIDSILNQTYDNFILYIRDDGSTDGTRKILKQYSEKDSRVKVQYGENIGYVKSFFKMLSEVNSEYIAFSDQDDIWLPEKLSVAQAALSQKNKSVPLMWASNIYICDEKMNVISIGARKRMSNFSNSLFMCNTQGMTMIINNKAREKVVSNLPKQNIMYHDWWIYRVVSAFGEVIFDSDPYVKYRRHDKNESDISYNFVNKVTNMMNRLINSDMYIRTKKETQEFKIIFDSQLSQSNRDVLSLFASPKRKIQKVFYSGRFKNSVLDELVLRLFFLLDIL

SEQ ID NO: 27 - protein, 473 aa, Lactococcus lactis subsp. lactis
MNNKLREGFTFTAIGTYSNFLIQIIVQAILSRLLSPREYGIIAIMQVFIVFFAMLVEAGMGPAIIQNKKLTNRDNMNLFNFSAIFSIIFAIIFGFLGLLLTKIYMNPAYTYLTWIQSISILFIGLNIVPTALLNKRKQFKAVNFSTVVGGILSGVVGVTMAFLGFGIYSLIASAITTAFVSFCLNRYFANIWFTKNWNKSSLISIWTVSRNQFGTNFINYFSNNSDNILVGKFMGDTALANYNKSYQLLTIPTTLLLNIVNPVLQPILSDYQDDVVTIRKTYYNIVHLLALIGIPTSIFLSMSAKQIIFFFFGSQWEEAVVPFSYLAVIVWCQMTTYSNGAIWQSRNKTNYFLFSSVINTFIIIFSIIIGIIIGNINAVALFVAIGNFISFFWKFYYITKNALEDSIRNLLKIFIHPIFLGFITFIGIRLEILIDPRNNFFSLLLRSLVFFSILITYIMFTSEKKIIEEIFDK

SEQ ID NO: 28 - protein, 388 aa, Lactococcus lactis subsp. lactis
MKIAVVGTGYVGLSISVLLAQHHEVVALDIVEAKVDLINSKKSPIVDKEIEGFLASKELNLLATTDTAQALNRADFVVIATPTNYDDVKNYFNTDSVEAVIEEVWKFSPNAMIVIKSTIPVGFVEKMRAKYDIDNIIFSPEFLREGRALYDNLHPSRIVVGEQSERASQFAELLIEGAIDKDIPVLFTNPTEAEAIKLFSNTYLALRVAYFNELDTYAEVRGLDTKQIIDGVGLDPRIGTHYNNPSFGYGGYCLPKDTKQLLANYDQVPEKLIEAVVESNSTRKDHIADMIIKRSPKVVGIYRLTMKSNSDNFRSSSIQGIMKRIKGKGIEVVVYEPTLNDTHFYNSRVVHNLDEFKTISDVIVSNRYTKELEDVKTKVYTRDLFGRD

SEQ ID NO: 29 - protein, 300 aa, Lactococcus lactis subsp. lactis
LERKKKKKKNIWVIIIPILIFITLIGAGAYALRDSLISTDHTKTNSSDQPTKTSASNGYVEKKGKEAAVGSIALVDDVGIPEWIKVPSKANLDKFTDLSTNNITIYRINNPEVLKTVTNRTDQRMKMSEVIAKYPNALIMNASAFDMQTGQVVGFQMNNGKLIQDWNPGTTTQYAFVINKDGSCKIYDSSTPASTIIKNGGQQAYDFGTAIIRDGKIQPSDGSVDWKIHIFIANDKDNNLYAILSDTNAGYDNIMKSVSNLKLQNMLLLDSGGSSQLSVNGKTIVASQDDRAVPDYIVMK

SEQ ID NO: 30 - protein, 300 aa, Lactococcus lactis subsp. lactis
MNQKKRRHYRKKKHTVLKVISIIFVLVIIAVASIAYVAYRNVESTFSTSYENFPKTTSIDLKKSKTFTTLIIATGKNNSKNTAYATVLASTNVKTNQTTFMNFPVFATMPNQKTITEVYNTNGDDGIFQMVKDLLNVSINKVIQIDVNKMGSLVQATGGITMQNPKAFNAEGYEFKQGTVNLQTADQVQAYMTQIDDTDLDASITRIQNVSMELYGNIQKVAHMKKLESFNYYREILYAFSNTVKTNISFNDAKTIVMSYNKALKNTGKLNLHTTDENGAKVVSQTELDSVKTLFEKSLK